European Patent Specification EP 3 365 062 B1, published September 18, 2024. Title: METHODS OF TREATING SOLID OR LYMPHATIC TUMORS BY COMBINATION THERAPY. Applicant: Cold Genesys, Inc. Application Not Yet Assigned. The sequence listing filed with the application follows.

SEQUENCE LISTING (1 sequence)

SEQ ID NO: 1 - DNA, 1519 bp, Homo sapiens
gggcccaaaattagcaagtgaccacgtggttctgaagccagtggcctaaggaccacccttgcagaaccgtggtctccttgtcacagtctaggcagcctctggcttagcctctgtttctttcataacctttctcagcgcctgctctgggccagaccagtgttgggaggagtcgctactgagctcctagattggcaggggaggcagatggagaaaaggagtgtgtgtggtcagcattggagcagaggcagcagtgggcaatagaggaagtgagtaaatccttgggagggctccctagaagtgatgtgttttctttttttgttttagagacaggatctcgctctgtcgcccaggctggtgtgcagtggcatgatcatagctcactgcagcctcgacttctcgggctcaagcaatcctcccacctcagcctcccaagtagctgggactacgggcacacgccaccatgcctggctaatttttgtattttttgtagagatgggtcttcaccatgttgatcaggctggtctcgaactcctgggctcatgcgatccaccccgccagctgattacagggattccggtggtgagccaccgcgcccagacgccacttcatcgtattgtaaacgtctgttacctttctgttcccctgtctactggactgtgagctccttagggccacgaattgaggatggggcacagagcaagctctccaaacgtttgttgaatgagtgagggaatgaatgagttcaagcagatgctatacgttggctgttggagattttggctaaaatgggacttgcaggaaagcccgacgtccccctcgccatttccaggcaccgctcttcagcttgggctctgggtgagcgggatagggctgggtgcaggattaggataatgtcatgggtgaggcaagttgaggatggaagaggtggctgatggctgggctgtggaactgatgatcctgaaaagaagaggggacagtctctggaaatctaagctgaggctgttgggggctacaggttgagggtcacgtgcagaagagaggctctgttctgaacctgcactatagaaaggtcagtgggatgcgggagcgtcggggcggggcggggcctatgttcccgtgtccccacgcctccagcaggggacgcccgggctgggggcggggagtcagaccgcgcctggtaccatccggacaaagcctgcgcgcgccccgccccgccattggccgtaccgccccgcgccgccgccccatcccgcccctcgccgccgggtccggcgcgttaaagccaataggaaccgccgccgttgttcccgtcacggacggggcagccaattgtggcggcgctcggcggctcgtggctctttcgcggcaaaaaggatttggcgcgtaaaagtggccgggactttgcaggcagcggcggccgggggcggagcgggatcgagccctcgccgaggcctgccgccatgggcccgcgccgccgccgccgcctgtcacccgggccgcgcgggccgtgagcgtcatg